European Patent Application EP 4 242 223 A2, published September 13, 2023. Title: MODIFIED MRNA VACCINES ENCODING HERPES SIMPLEX VIRUS GLYCOPROTEINS AND USES THEREOF. Applicant: The Trustees of The University of Pennsylvania. Application EP. The sequence listing filed with the application follows.

SEQUENCE LISTING (18 sequences)

SEQ ID NO: 1 - RNA, 1386 nt, synthetic construct
  misc_feature 1..1386: note = All uridine residues are 1-methyl-pseudouridine - encodes glycoprotein D from Herpes Simplex Virus-1
  source 1..1386: mol_type = other RNA
ggaataaaagtctcaacacaacatatacaaaacaaacgaatctcaagcaatcaagcattctacttctattgcagcaatttaaatcatttcttttaaagcaaaagcaattttctgaaaattttcaccatttacgaacgatagcatgcgcatgcagctgctgctgctgatcgccctgtccctggccctggtgaccaactccaagtacgccctggccgacgcctccctgaagatggccgaccccaaccgcttccgcggcaaggacctgcccgtgctggaccagctgaccgacccccccggcgtgcgccgcgtgtaccacatccaggccggcctgcccgaccccttccagcccccctccctgcccatcaccgtgtactacgccgtgctggagcgcgcctgccgctccgtgctgctgaacgccccctccgaggccccccagatcgtgcgcggcgcctccgaggacgtgcgcaagcagccctacaacctgaccatcgcctggttccgcatgggcggcaactgcgccatccccatcaccgtgatggagtacaccgagtgctcctacaacaagtccctgggcgcctgccccatccgcacccagccccgctggaactactacgactccttctccgccgtgtccgaggacaacctgggcttcctgatgcacgcccccgccttcgagaccgccggcacctacctgcgcctggtgaagatcaacgactggaccgagatcacccagttcatcctggagcaccgcgccaagggctcctgcaagtacgccctgcccctgcgcatccccccctccgcctgcctgtccccccaggcctaccagcagggcgtgaccgtggactccatcggcatgctgccccgcttcatccccgagaaccagcgcaccgtggccgtgtactccctgaagatcgccggctggcacggccccaaggccccctacacctccaccctgctgccccccgagctgtccgagacccccaacgccacccagcccgagctggcccccgaggaccccgaggactccgccctgctggaggaccccgtgggcaccgtggccccccagatcccccccaactggcacatcccctccatccaggacgccgccaccccctactaactagtagtgactgactaggatctggttaccactaaaccagcctcaagaacacccgaatggagtctctaagctacataataccaacttacacttacaaaatgttgtcccccaaaatgtagccattcgtatctgctcctaataaaaagaaagtttcttcacattctaaaaaaaaaaaaaaaaaaaaaaaaaaaaaaaaaaaaaaaaaaaaaaaaaaaaaaaaaaaaaaaaaaaaaaaaaaaaaaaaaaaaaaaaaaaaaaaaaaaaac

SEQ ID NO: 2 - protein, 306 aa, Human alphaherpesvirus 1
KYALADASLKMADPNRFRGKDLPVLDQLTDPPGVRRVYHIQAGLPDPFQPPSLPITVYYAVLERACRSVLLNAPSEAPQIVRGASEDVRKQPYNLTIAWFRMGGNCAIPITVMEYTECSYNKSLGACPIRTQPRWNYYDSFSAVSEDNLGFLMHAPAFETAGTYLRLVKINDWTEITQFILEHRAKGSCKYALPLRIPPSACLSPQAYQQGVTVDSIGMLPRFIPENQRTVAVYSLKIAGWHGPKAPYTSTLLPPELSETPNATQPELAPEDPEDSALLEDPVGTVAPQIPPNWHIPSIQDAATPY

SEQ ID NO: 3 - protein, 394 aa, Human alphaherpesvirus 1
MGGAAARLGAVILFVVIVGLHGVRGKYALADASLKLADPNRFRRKDLPVLDQLTDPPGVRRVYHIQAGLPDPFQPPSLPITVYYAVLERACRSVLLNAPSEAPQIVRGASEDVRKQPYNLTIAWFRMGGNCAIPITVMEYTECSYNKSLGACPIRTQPRWNYYDSFSAVSEDNLGFLMHAPAFETAGTYLRLVKINDWTEITQFILEHRAKGSCKYALPLRIPPSACLSPQAYQQGVTVDSIGMLPRFIPENQRTVAVYSLKIAGWHGPKAPYTSTLLPPELSETPNATQPELAPEAPEDSALLEDPVGTVAPQIPPNWHIPSIQDAATPYHPPATPNNMGLIAGAVGGSLLAALVICGIVYWMRRRTQKAPKRIRLPHIREDDQPSSHQPLFY

SEQ ID NO: 4 - RNA, 1386 nt, synthetic construct
  misc_feature 1..1386: note = All uridine residues are 1-methyl-pseudouridine - encodes glycoprotein D from Herpes Simplex Virus-2
  source 1..1386: mol_type = other RNA
ggaataaaagtctcaacacaacatatacaaaacaaacgaatctcaagcaatcaagcattctacttctattgcagcaatttaaatcatttcttttaaagcaaaagcaattttctgaaaattttcaccatttacgaacgatagcatgacccgcctgaccgtgctggccctgctggccggcctgctggcctcctcccgcgccaagtacgccctggccgacccctccctgaagatggccgaccccaaccgcttccgcggcaagaacctgcccgtgctggaccagctgaccgacccccccggcgtgaagcgcgtgtaccacatccagccctccctggaggaccccttccagcccccctccatccccatcaccgtgtactacgccgtgctggagcgcgcctgccgctccgtgctgctgcacgccccctccgaggccccccagatcgtgcgcggcgcctccgacgaggcccgcaagcacacctacaacctgaccatcgcctggtaccgcatgggcgacaactgcgccatccccatcaccgtgatggagtacaccgagtgcccctacaacaagtccctgggcgtgtgccccatccgcacccagccccgctggtcctactacgactccttctccgccgtgtccgaggacaacctgggcttcctgatgcacgcccccgccttcgagaccgccggcacctacctgcgcctggtgaagatcaacgactggaccgagatcacccagttcatcctggagcaccgcgcccgcgcctcctgcaagtacgccctgcccctgcgcatcccccccgccgcctgcctgacctccaaggcctaccagcagggcgtgaccgtggactccatcggcatgctgccccgcttcatccccgagaaccagcgcaccgtggccctgtactccctgaagatcgccggctggcacggccccaagcccccctacacctccaccctgctgccccccgagctgtccgacaccaccaacgccacccagcccgagctggtgcccgaggaccccgaggactccgccctgctggaggaccccgccggcaccgtgtcctcccagatcccccccaactggcacatcccctccatccaggacgtggccccccaccactaactagtagtgactgactaggatctggttaccactaaaccagcctcaagaacacccgaatggagtctctaagctacataataccaacttacacttacaaaatgttgtcccccaaaatgtagccattcgtatctgctcctaataaaaagaaagtttcttcacattctaaaaaaaaaaaaaaaaaaaaaaaaaaaaaaaaaaaaaaaaaaaaaaaaaaaaaaaaaaaaaaaaaaaaaaaaaaaaaaaaaaaaaaaaaaaaaaaaaaaaac

SEQ ID NO: 5 - protein, 306 aa, Human alphaherpesvirus 2
KYALADPSLKMADPNRFRGKNLPVLDQLTDPPGVKRVYHIQPSLEDPFQPPSIPITVYYAVLERACRSVLLHAPSEAPQIVRGASDEARKHTYNLTIAWYRMGDNCAIPITVMEYTECPYNKSLGVCPIRTQPRWSYYDSFSAVSEDNLGFLMHAPAFETAGTYLRLVKINDWTEITQFILEHRARASCKYALPLRIPPAACLTSKAYQQGVTVDSIGMLPRFIPENQRTVALYSLKIAGWHGPKPPYTSTLLPPELSDTTNATQPELVPEDPEDSALLEDPAGTVSSQIPPNWHIPSIQDVAPHH

SEQ ID NO: 6 - protein, 393 aa, Human alphaherpesvirus 2
MGRLTSGVGTAALLVVAVGLRVVCAKYALADPSLKMADPNRFRGKNLPVLDQLTDPPGVKRVYHIQPSLEDPFQPPSIPITVYYAVLERACRSVLLHAPSEAPQIVRGASDEARKHTYNLTIAWYRMGDNCAIPITVMEYTECPYNKSLGVCPIRTQPRWSYYDSFSAVSEDNLGFLMHAPAFETAGTYLRLVKINDWTEITQFILEHRARASCKYALPLRIPPAACLTSKAYQQGVTVDSIGMLPRFIPENQRTVALYSLKIAGWHGPKPPYTSTLLPPELSDTTNATQPELVPEDPEDSALLEDPAGTVSSQIPPNWHIPSIQDVAPHHAPAAPSNPGLIIGALAGSTLAVLVIGGIAFWVRRRAQMAPKRLRLPHIRDDDAPPSHQPLFY

SEQ ID NO: 7 - RNA, 1779 nt, synthetic construct
  misc_feature 1..1779: note = All uridine residues are 1-methyl-pseudouridine - encodes glycoprotein C from Herpes Simplex Virus-1
  source 1..1779: mol_type = other RNA
ggaataaaagtctcaacacaacatatacaaaacaaacgaatctcaagcaatcaagcattctacttctattgcagcaatttaaatcatttcttttaaagcaaaagcaattttctgaaaattttcaccatttacgaacgatagcatggccatctccggcgtgcccgtgctgggcttcttcatcatcgccgtgctgatgtccgcccaggagtcctgggccgagaccgcctccaccggccccaccatcaccgccggcgccgtgaccaacgcctccgaggcccccacctccggctcccccggctccgccgcctcccccgaggtgacccccacctccacccccaaccccaacaacgtgacccagaacaagaccacccccaccgagcccgcctccccccccaccacccccaagcccacctccacccccaagtccccccccacctccacccccgaccccaagcccaagaacaacaccacccccgccaagtccggccgccccaccaagccccccggccccgtgtggtgcgaccgccgcgaccccctggcccgctacggctcccgcgtgcagatccgctgccgcttccgcaactccacccgcatggagttccgcctgcagatctggcgctactccatgggcccctccccccccatcgcccccgcccccgacctggaggaggtgctgaccaacatcaccgccccccccggcggcctgctggtgtacgactccgcccccaacctgaccgacccccacgtgctgtgggccgagggcgccggccccggcgccgacccccccctgtactccgtgaccggccccctgcccacccagcgcctgatcatcggcgaggtgacccccgccacccagggcatgtactacctggcctggggccgcatggactccccccacgagtacggcacctgggtgcgcgtgcgcatgttccgccccccctccctgaccctgcagccccacgccgtgatggagggccagcccttcaaggccacctgcaccgccgccgcctactacccccgcaaccccgtggagttcgactggttcgaggacgaccgccaggtgttcaaccccggccagatcgacacccagacccacgagcaccccgacggcttcaccaccgtgtccaccgtgacctccgaggccgtgggcggccaggtgcccccccgcaccttcacctgccagatgacctggcaccgcgactccgtgaccttctcccgccgcaacgccaccggcctggccctggtgctgccccgccccaccatcaccatggagttcggcgtgcgccacgtggtgtgcaccgccggctgcgtgcccgagggcgtgaccttcgcctggttcctgggcgacgacccctcccccgccgccaagtccgccgtgaccgcccaggagtcctgcgaccaccccggcctggccaccgtgcgctccaccctgcccatctcctacgactactccgagtacatctgccgcctgaccggctaccccgccggcatccccgtgctggagcaccactaactagtagtgactgactaggatctggttaccactaaaccagcctcaagaacacccgaatggagtctctaagctacataataccaacttacacttacaaaatgttgtcccccaaaatgtagccattcgtatctgctcctaataaaaagaaagtttcttcacattctaaaaaaaaaaaaaaaaaaaaaaaaaaaaaaaaaaaaaaaaaaaaaaaaaaaaaaaaaaaaaaaaaaaaaaaaaaaaaaaaaaaaaaaaaaaaaaaaaaaaac

SEQ ID NO: 8 - protein, 431 aa, Human alphaherpesvirus 1
ETASTGPTITAGAVTNASEAPTSGSPGSAASPEVTPTSTPNPNNVTQNKTTPTEPASPPTTPKPTSTPKSPPTSTPDPKPKNNTTPAKSGRPTKPPGPVWCDRRDPLARYGSRVQIRCRFRNSTRMEFRLQIWRYSMGPSPPIAPAPDLEEVLTNITAPPGGLLVYDSAPNLTDPHVLWAEGAGPGADPPLYSVTGPLPTQRLIIGEVTPATQGMYYLAWGRMDSPHEYGTWVRVRMFRPPSLTLQPHAVMEGQPFKATCTAAAYYPRNPVEFDWFEDDRQVFNPGQIDTQTHEHPDGFTTVSTVTSEAVGGQVPPRTFTCQMTWHRDSVTFSRRNATGLALVLPRPTITMEFGVRHVVCTAGCVPEGVTFAWFLGDDPSPAAKSAVTAQESCDHPGLATVRSTLPISYDYSEYICRLTGYPAGIPVLEHH

SEQ ID NO: 9 - protein, 511 aa, Human alphaherpesvirus 1
MAPGRVGLAVVLWGLLWLGAGVAGGSETASTGPTITAGAVTNASEAPTSGSPGSAASPEVTPTSTPNPNNVTQNKTTPTEPASPPTTPKPTSTPKSPPTSTPDPKPKNNTTPAKSGRPTKPPGPVWCDRRDPLARYGSRVQIRCRFRNSTRMEFRLQIWRYSMGPSPPIAPAPDLEEVLTNITAPPGGLLVYDSAPNLTDPHVLWAEGAGPGADPPLYSVTGPLPTQRLIIGEVTPATQGMYYLAWGRMDSPHEYGTWVRVRMFRPPSLTLQPHAVMEGQPFKATCTAAAYYPRNPVEFDWFEDDRQVFNPGQIDTQTHEHPDGFTTVSTVTSEAVGGQVPPRTFTCQMTWHRDSVTFSRRNATGLALVLPRPTITMEFGVRHVVCTAGCVPEGVTFAWFLGDDPSPAAKSAVTAQESCDHPGLATVRSTLPISYDYSEYICRLTGYPAGIPVLEHHGSHQPPPRDPTERQVIEAIEWVGIGIGVLAAGVLVVTAIVYVVRTSQSRQRHRR

SEQ ID NO: 10 - RNA, 1668 nt, synthetic construct
  misc_feature 1..1668: note = All uridine residues are 1-methyl-pseudouridine - encodes glycoprotein C from Herpes Simplex Virus-2
  source 1..1668: mol_type = other RNA
ggaataaaagtctcaacacaacatatacaaaacaaacgaatctcaagcaatcaagcattctacttctattgcagcaatttaaatcatttcttttaaagcaaaagcaattttctgaaaattttcaccatttacgaacgatagcatgcgcatgcagctgctgctgctgatcgccctgtccctggccctggtgaccaactccgcctcccccggccgcaccatcaccgtgggcccccgcggcaacgcctccaacgccgccccctccgcctccccccgcaacgcctccgccccccgcaccacccccacccccccccagccccgcaaggccaccaagtccaaggcctccaccgccaagcccgcccccccccccaagaccggcccccccaagacctcctccgagcccgtgcgctgcaaccgccacgaccccctggcccgctacggctcccgcgtgcagatccgctgccgcttccccaactccacccgcaccgagttccgcctgcagatctggcgctacgccaccgccaccgacgccgagatcggcaccgccccctccctggaggaggtgatggtgaacgtgtccgccccccccggcggccagctggtgtacgactccgcccccaaccgcaccgacccccacgtgatctgggccgagggcgccggccccggcgcctccccccgcctgtactccgtggtgggccccctgggccgccagcgcctgatcatcgaggagctgaccctggagacccagggcatgtactactgggtgtggggccgcaccgaccgcccctccgcctacggcacctgggtgcgcgtgcgcgtgttccgccccccctccctgaccatccacccccacgccgtgctggagggccagcccttcaaggccacctgcaccgccgccacctactaccccggcaaccgcgccgagttcgtgtggttcgaggacggccgccgcgtgttcgaccccgcccagatccacacccagacccaggagaaccccgacggcttctccaccgtgtccaccgtgacctccgccgccgtgggcggccagggccccccccgcaccttcacctgccagctgacctggcaccgcgactccgtgtccttctcccgccgcaacgcctccggcaccgcctccgtgctgccccgccccaccatcaccatggagttcaccggcgaccacgccgtgtgcaccgccggctgcgtgcccgagggcgtgaccttcgcctggttcctgggcgacgactcctcccccgccgagaaggtggccgtggcctcccagacctcctgcggccgccccggcaccgccaccatccgctccaccctgcccgtgtcctacgagcagaccgagtacatctgccgcctggccggctaccccgacggcatccccgtgctggagcaccactaactagtagtgactgactaggatctggttaccactaaaccagcctcaagaacacccgaatggagtctctaagctacataataccaacttacacttacaaaatgttgtcccccaaaatgtagccattcgtatctgctcctaataaaaagaaagtttcttcacattctaaaaaaaaaaaaaaaaaaaaaaaaaaaaaaaaaaaaaaaaaaaaaaaaaaaaaaaaaaaaaaaaaaaaaaaaaaaaaaaaaaaaaaaaaaaaaaaaaaaaac

SEQ ID NO: 11 - protein, 400 aa, Human alphaherpesvirus 2
ASPGRTITVGPRGNASNAAPSASPRNASAPRTTPTPPQPRKATKSKASTAKPAPPPKTGPPKTSSEPVRCNRHDPLARYGSRVQIRCRFPNSTRTESRLQIWRYATATDAEIGTAPSLEEVMVNVSAPPGGQLVYDSAPNRTDPHVIWAEGAGPGASPRLYSVVGPLGRQRLIIEELTLETQGMYYWVWGRTDRPSAYGTWVRVRVFRPPSLTIHPHAVLEGQPFKATCTAATYYPGNRAEFVWFEDGRRVFDPAQIHTQTQENPDGFSTVSTVTSAAVGGQGPPRTFTCQLTWHRDSVSFSRRNASGTASVLPRPTITMEFTGDHAVCTAGCVPEGVTFAWFLGDDSSPAEKVAVASQTSCGRPGTATIRSTLPVSYEQTEYICRLAGYPDGIPVLEHH

SEQ ID NO: 12 - protein, 480 aa, Human alphaherpesvirus 2
MALGRVGLAVGLWGLLWVGVVVVLANASPGRTITVGPRGNASNAAPSASPRNASAPRTTPTPPQPRKATKSKASTAKPAPPPKTGPPKTSSEPVRCNRHDPLARYGSRVQIRCRFPNSTRTEFRLQIWRYATATDAEIGTAPSLEEVMVNVSAPPGGQLVYDSAPNRTDPHVIWAEGAGPGASPRLYSVVGPLGRQRLIIEELTLETQGMYYWVWGRTDRPSAYGTWVRVRVFRPPSLTIHPHAVLEGQPFKATCTAATYYPGNRAEFVWFEDGRRVFDPAQIHTQTQENPDGFSTVSTVTSAAVGGQGPPRTFTCQLTWHRDSVSFSRRNASGTASVLPRPTITMEFTGDHAVCTAGCVPEGVTFAWFLGDDSSPAEKVAVASQTSCGRPGTATIRSTLPVSYEQTEYICRLAGYPDGIPVLEHHGSHQPPPRDPTERQVIRAVEGAGIGVAVLVAVVLAGTAVVYLTHASSVRYRRLR

SEQ ID NO: 13 - RNA, 1626 nt, synthetic construct
  misc_feature 1..1626: note = All uridine residues are 1-methyl-pseudouridine - encodes glycoprotein E from Herpes Simplex Virus-1
  source 1..1626: mol_type = other RNA
ggaataaaagtctcaacacaacatatacaaaacaaacgaatctcaagcaatcaagcattctacttctattgcagcaatttaaatcatttcttttaaagcaaaagcaattttctgaaaattttcaccatttacgaacgatagcatgcgcatgcagctgctgctgctgatcgccctgtccctggccctggtgaccaactccaagacctcctggcgccgcgtgtccgtgggcgaggacgtgtccctgctgcccgcccccggccccaccggccgcggccccacccagaagctgctgtgggccgtggagcccctggacggctgcggccccctgcacccctcctgggtgtccctgatgccccccaagcaggtgcccgagaccgtggtggacgccgcctgcatgcgcgcccccgtgcccctggccatggcctacgccccccccgccccctccgccaccggcggcctgcgcaccgacttcgtgtggcaggagcgcgccgccgtggtgaaccgctccctggtgatctacggcgtgcgcgagaccgactccggcctgtacaccctgtccgtgggcgacatcaaggaccccgcccgccaggtggcctccgtggtgctggtggtgcagcccgcccccgtgcccacccccccccccacccccgccgactacgacgaggacgacaacgacgagggcgagggcgaggacgagtccctggccggcacccccgcctccggcaccccccgcctgcccccctcccccgcccccccccgctcctggccctccgcccccgaggtgtcccacgtgcgcggcgtgaccgtgcgcatggagacccccgaggccatcctgttctcccccggcgaggccttctccaccaacgtgtccatccacgccatcgcccacgacgaccagacctacaccatggacgtggtgtggctgcgcttcgacgtgcccacctcctgcgccgagatgcgcatctacgagtcctgcctgtaccacccccagctgcccgagtgcctgtcccccgccgacgccccctgcgccgcctccacctggacctcccgcctggccgtgcgctcctacgccggctgctcccgcaccaacccccccccccgctgctccgccgaggcccacatggagcccttccccggcctggcctggcaggccgcctccgtgaacctggagttccgcgacgcctccccccagcactccggcctgtacctgtgcgtggtgtacgtgaacgaccacatccacgcctggggccacatcaccatcaacaccgccgcccagtaccgcaacgccgtggtggagcagcccctgccccagcgcggcgccgacctggccgagcccacccacccccacgtgggcgcctaactagtagtgactgactaggatctggttaccactaaaccagcctcaagaacacccgaatggagtctctaagctacataataccaacttacacttacaaaatgttgtcccccaaaatgtagccattcgtatctgctcctaataaaaagaaagtttcttcacattctaaaaaaaaaaaaaaaaaaaaaaaaaaaaaaaaaaaaaaaaaaaaaaaaaaaaaaaaaaaaaaaaaaaaaaaaaaaaaaaaaaaaaaaaaaaaaaaaaaaaac

SEQ ID NO: 14 - protein, 386 aa, Human alphaherpesvirus 1
KTSWRRVSVGEDVSLLPAPGPTGRGPTQKLLWAVEPLDGCGPLHPSWVSLMPPKQVPETVVDAACMRAPVPLAMAYAPPAPSATGGLRTDFVWQERAAVVNRSLVIYGVRETDSGLYTLSVGDIKDPARQVASVVLVVQPAPVPTPPPTPADYDEDDNDEGEGEDESLAGTPASGTPRLPPSPAPPRSWPSAPEVSHVRGVTVRMETPEAILFSPGEAFSTNVSIHAIAHDDQTYTMDVVWLRFDVPTSCAEMRIYESCLYHPQLPECLSPADAPCAASTWTSRLAVRSYAGCSRTNPPPRCSAEAHMEPFPGLAWQAASVNLEFRDASPQHSGLYLCVVYVNDHIHAWGHITINTAAQYRNAVVEQPLPQRGADLAEPTHPHVGA

SEQ ID NO: 15 - protein, 552 aa, Human alphaherpesvirus 1
MDRGAVVGFLLGVCVVSCLAGTPKTSWRRVSVGEDVSLLPAPGPTGRGPTQKLLWAVEPLDGCGPLHPSWVSLMPPKQVPETVVDAACMRAPVPLAMAYAPPAPSATGGLRTDFVWQERAAVVNRSLVIYGVRETDSGLYTLSVGDIKDPARQVASVVLVVQPAPVPTPPPTPADYDEDDNDEGEGEDESLAGTPASGTPRLPPSPAPPRSWPSAPEVSHVRGVTVRMETPEAILFSPGEAFSTNVSIHAIAHDDQTYTMDVVWLRFDVPTSCAEMRIYESCLYHPQLPECLSPADAPCAASTWTSRLAVRSYAGCSRTNPPPRCSAEAHMEPFPGLAWQAASVNLEFRDASPQHSGLYLCVVYVNDHIHAWGHITINTAAQYRNAVVEQPLPQRGADLAEPTHPHVGAPPHAPPTHGALRLGAVMGAALLLSALGLSVWACMTCWRRRAWRAVKSRASGKGPTYIRVADSELYADWSSDSEGERDQVPWLAPPERPDSPSTNGSGFEILSPTAPSVYPRSDGHQSRRQLTTFGSGRPDRRYSQASDSSVFW

SEQ ID NO: 16 - RNA, 1614 nt, synthetic construct
  misc_feature 1..1614: note = All uridine residues are 1-methyl-pseudouridine - encodes glycoprotein E from Herpes Simplex Virus-2
  source 1..1614: mol_type = other RNA
ggaataaaagtctcaacacaacatatacaaaacaaacgaatctcaagcaatcaagcattctacttctattgcagcaatttaaatcatttcttttaaagcaaaagcaattttctgaaaattttcaccatttacgaacgatagcatgcgcatgcagctgctgctgctgatcgccctgtccctggccctggtgaccaactcccgcacctcctggaagcgcgtgacctccggcgaggacgtggtgctgctgcccgcccccgccggccccgaggagcgcacccgcgcccacaagctgctgtgggccgccgagcccctggacgcctgcggccccctgcgcccctcctgggtggccctgtggcccccccgccgcgtgctggagaccgtggtggacgccgcctgcatgcgcgcccccgagcccctggccatcgcctactccccccccttccccgccggcgacgagggcctgtactccgagctggcctggcgcgaccgcgtggccgtggtgaacgagtccctggtgatctacggcgccctggagaccgactccggcctgtacaccctgtccgtggtgggcctgtccgacgaggcccgccaggtggcctccgtggtgctggtggtggagcccgcccccgtgcccacccccacccccgacgactacgacgaggaggacgacgccggcgtgtccgagcgcacccccgtgtccgtgcccccccccacccccccccgccgcccccccgtggccccccccacccacccccgcgtgatccccgaggtgtcccacgtgcgcggcgtgaccgtgcacatggagacccccgaggccatcctgttcgcccccggcgagaccttcggcaccaacgtgtccatccacgccatcgcccacgacgacggcccctacgccatggacgtggtgtggatgcgcttcgacgtgccctcctcctgcgccgagatgcgcatctacgaggcctgcctgtaccacccccagctgcccgagtgcctgtcccccgccgacgccccctgcgccgtgtcctcctgggcctaccgcctggccgtgcgctcctacgccggctgctcccgcaccaccccccccccccgctgcttcgccgaggcccgcatggagcccgtgcccggcctggcctggctggcctccaccgtgaacctggagttccagcacgcctccccccagcacgccggcctgtacctgtgcgtggtgtacgtggacgaccacatccacgcctggggccacatgaccatctccaccgccgcccagtaccgcaacgccgtggtggagcagcacctgccccagcgccagcccgagcccgtggagcccacccgcccccacgtgcgcgcctaactagtagtgactgactaggatctggttaccactaaaccagcctcaagaacacccgaatggagtctctaagctacataataccaacttacacttacaaaatgttgtcccccaaaatgtagccattcgtatctgctcctaataaaaagaaagtttcttcacattctaaaaaaaaaaaaaaaaaaaaaaaaaaaaaaaaaaaaaaaaaaaaaaaaaaaaaaaaaaaaaaaaaaaaaaaaaaaaaaaaaaaaaaaaaaaaaaaaaaaaac

SEQ ID NO: 17 - protein, 382 aa, Human alphaherpesvirus 2
RTSWKRVTSGEDVVLLPAPAGPEERTRAHKLLWAAEPLDACGPLRPSWVALWPPRRVLETVVDAACMRAPEPLAIAYSPPFPAGDEGLYSELAWRDRVAVVNESLVIYGALETDSGLYTLSVVGLSDEARQVASVVLVVEPAPVPTPTPDDYDEEDDAGVSERTPVSVPPPTPPRRPPVAPPTHPRVIPEVSHVRGVTVHMETPEAILFAPGETFGTNVSIHAIAHDDGPYAMDVVWMRFDVPSSCAEMRIYEACLYHPQLPECLSPADAPCAVSSWAYRLAVRSYAGCSRTTPPPRCFAEARMEPVPGLAWLASTVNLEFQHASPQHAGLYLCVVYVDDHIHAWGHMTISTAAQYRNAVVEQHLPQRQPEPVEPTRPHVRA

SEQ ID NO: 18 - protein, 545 aa, Human alphaherpesvirus 2
MARGAGLVFFVGVWVVSCLAAAPRTSWKRVTSGEDVVLLPAPAERTRAHKLLWAAEPLDACGPLRPSWVALWPPRRVLETVVDAACMRAPEPLAIAYSPPFPAGDEGLYSELAWRDRVAVVNESLVIYGALETDSGLYTLSVVGLSDEARQVASVVLVVEPAPVPTPTPDDYDEEDDAGVTNARRSAFPPQPPPRRPPVAPPTHPRVIPEVSHVRGVTVHMETLEAILFAPGETFGTNVSIHAIAHDDGPYAMDVVWMRFDVPSSCADMRIYEACLYHPQLPECLSPADAPCAVSSWAYRLAVRSYAGCSRTTPPPRCFAEARMEPVPGLAWLASTVNLEFQHASPQHAGLYLCVVYVDDHIHAWGHMTISTAAQYRNAVVEQHLPQRQPEPVEPTRPHVRAPHPAPSARGPLRLGAVLGAALLLAALGLSAWACMTCWRRRSWRAVKSRASATGPTYIRVADSELYADWSSDSEGERDGSLWQDPPERPDSPSTNGSGFEILSPTAPSVYPHSEGRKSRRPLTTFGSGSPGRRHSQASYPSVLW